European Patent Application EP 4 600 362 A1, published August 13, 2025. Title: REPORTER GENE CONSTRUCT SENSITIVE TO QUEUOSINE LEVELS. Applicant: INSTITUTO NACIONAL DE TECNICA AEROESPACIAL. The sequence listing filed with the application follows.

SEQUENCE LISTING (1 sequence)

SEQ ID NO: 1 - DNA, 1310 bp, synthetic construct
  source 1..1310: mol_type = other DNA
ctcctcttttgtacagttcattgtacaatgatgagcgttaattaactatttattaattagtttgtagatcaaggtattgtcagtgagacgaaaatccaggcttcgctatttttggtgccatcagctaagaggacagtcctcttagccccctcctttccccgctcattcattaaacaaatccattgccataaaatatataaaaaagcccttgctttctaacgtgaaagtggtttaggttaaaagacatcagttgaataaacattcacagagacttttatgacacgcgttcaatttaaacaccaccatcatcaccatcatcctgactagtctttcaggcgatgtgtgctggaagacattcagatcttccagtggtgcatgaacgcatgagaaagcccccggaagatcaccttccgggggcttttttattgcgcggttgataacggttcagacaggtttaaagaggaataacaaaatgacagacaacactgtgagcaagggcgaggagctgttcaccggggtggtgcccatcctggtcgagctggacggcgacgtaaacggccacaagttcagcgtgtccggcgagggcgagggcgacgccacctacggcaagctgaccctgaagttcatctgcaccaccggcaagctgcccgtgccctggcccaccctcgtgaccaccctgacctacggcgtgcagtgcttcagccgctaccccgaccacatgaagcagcacgacttcttcaagtccgccatgcccgaaggctacgtccaggagcgcaccatcttcttcaaggacgacggcaactacaagacccgcgccgaggtgaagttcgagggcgacaccctggtgaaccgcatcgagctgaagggcatcgacttcaaggaggacggcaacatcctggggcacaagctggagtacaactacaacagccacaacgtctacatcatggccgacaagcagaagaacggcatcaaggtgaacttcaagatccgccacaacatcgaggacggcagcgtgcagctcgccgaccactaccagcagaacacccccatcggcgacggccccgtgctgctgcccgacaaccactacctgagcacccagtccgccctgagcaaagaccccaacgagaagcgcgaccacatggtcctgctggagttcgtgaccgccgccgggatcactctcggcatggacgagctgtacaagtaatcgcttggactcctgttgatagatccagtaatgacctcagaactccatctggatttgttcagaacgctcggttgccgccgggcgttttttattggtgagaatccaa